European Patent Specification EP 3 369 811 B1, published September 3, 2025. Title: METHOD FOR PRODUCING PANCREATIC ENDOCRINE CELLS, AND TRANS-DIFFERENTIATION AGENT. Applicant: Saitama Medical University. The sequence listing filed with the application follows.

SEQUENCE LISTING (10 sequences)

SEQ ID NO: 1 - DNA, 1290 bp, Artificial Sequence
  Artificial Sequence
atggttgccggtcggcaggcatgccgctgggtggactgctgcgcagcctacgagcagcaggaggagctggtgcggcacatcgagaagagccacatcgaccagcgcaagggcgaagacttcacctgcttctgggccgggtgtgtgcggcgctacaagcccttcaatgcccgctacaagctgctcatccacatgagggtacactcaggcgagaagcccaacaagtgcatgttcgaaggctgcagtaaagccttttcccgtctggagaacctgaagatccatctgcggagccacacaggcgagaaaccatacctgtgccagcacccaggctgccagaaggccttcagcaactccagcgaccgtgccaagcaccaacgcacccacctcgacacgaagccatatgcttgtcagatccctggctgctccaagcgctacacggaccccagctccctccgcaagcacgtgaaggcccactcagccaaagagcagcaggtgcgtaagaagctgcacacaggtgccgacccagaggctgatgttctgtccgagtgtctgtccctgcagcagctccaagcatccacactgttgccggccagcagagggaagggcagccaaaccctgagccaggagctcctcccaggtgtgtatcctggctccgtcaccccacaaaacgggcttgcttcaggcatcctgtccccctcccacgatgtcccttccaggcaccacccactggaggtccccactggttcccaccaccacctgtcccctctgcccacagctgagagcaccagggatggcctggggcccagtctcctttcacccatggtcagcccactgaaggggcttggtcccccaccgctaccaccagcctcccagagtcagtctccagggggacagtcattctctacagtccccagcaagcctacctacccatccttccaaagcccaccacctctgcccagcccccaaggctaccaaggcagtttccattccatccagaactgcttcccctacgctgactgctaccgggccactgagccagcagcctccagggatggactggtgggtgatgcccacggtttcaaccccttgcgacccagcacatactccagcctcagcacacctttatccgcaccaggctacgagaccctggcagaaacgccgtgtcccccagcgctgcagccacagccagctgaagacctggtacctagtggtcctgaggactgtggcttcttccccaatggggcctttgaccactgtctgagtcacatcccgtccatctacactgacacctga

SEQ ID NO: 2 - DNA, 1299 bp, Artificial Sequence
  Artificial Sequence
atggtggtggccgggcggcaggcgtgccgctgggtggactgctgtgcagcctatgagcagcaggaggagctggtgcggcacatcgagaagagccacatcgaccagcgcaagggcgaggacttcacctgcttctgggctggctgcgtgcgccgctacaagcccttcaacgcccgctacaagctgctcatccacatgcgagtgcactcgggcgagaagcccaacaagtgcatgtttgaaggctgcagcaaggccttctcacggctggagaacctcaagatccacctgaggagccacacgggcgagaagccgtacctgtgccagcacccgggttgccagaaggccttcagcaactccagcgaccgcgccaagcaccagcgcacccacctagacacgaagccgtacgcctgtcagatccctggctgctccaagcgctacacagaccccagctccctccgcaagcacgtcaaggcccattcagccaaagagcagcaggtgcgtaagaagctgcatgcgggccctgacaccgaggccgacgtcctgaccgagtgtctggtcctgcagcagctccacacgtccacacagctggctgccagcgacggcaagggtggctgtggcctgggccaggagctgctcccaggtgtgtatcctggctccatcaccccccataacggacttgcatcgggcctcctgcccccagcgcacgacgtaccttccaggcaccacccgctggatgccaccaccagttcccaccaccatctgtcccctctgcccatggctgagagcacccgggatgggttggggcccggcctcctctcaccaatagtcagccccctgaaggggctggggccaccgccgctgcccccatcctctcagagccattctccggggggccagcccttccccacactccccagcaagccgtcctacccacccttccagagccctccacccccgcctctgcccagcccacaaggttaccagggcagtttccactccatccagagttgcttcccctatggcgactgctaccggatggctgaaccagcagccggtggggacggactggtcggggagacccacggtttcaaccccctgcggcccaatggctaccacagcctcagcacgcccttgcctgccacaggctatgaggccctggctgaggcctcatgccccacagcgctgccacagcagccatctgaagatgtggtgtccagcggccccgaggactgtggcttcttccccaatggagcctttgaccactgcctgggccacatcccctccatctacacagacacctga

SEQ ID NO: 3 - DNA, 21 bp, Artificial Sequence
  primer
tggagaaacctgccaagtatg

SEQ ID NO: 4 - DNA, 20 bp, Artificial Sequence
  primer
ggagacaacctggtcctcag

SEQ ID NO: 5 - DNA, 20 bp, Artificial Sequence
  primer
tttgtcaagcagcacctttg

SEQ ID NO: 6 - DNA, 20 bp, Artificial Sequence
  primer
ggtctgaaggtcacctgctc

SEQ ID NO: 7 - DNA, 20 bp, Artificial Sequence
  primer
atgttcgtcatgggtgtgaa

SEQ ID NO: 8 - DNA, 20 bp, Artificial Sequence
  primer
tgtggtcatgagtccttcca

SEQ ID NO: 9 - DNA, 20 bp, Artificial Sequence
  primer
gccatcaagcagatcactgt

SEQ ID NO: 10 - DNA, 20 bp, Artificial Sequence
  primer
caggtgttggttcacaaagg